European Patent Application EP 4 273 237 A1, published November 8, 2023. Title: Transaminase mutants and uses thereof. Applicant: ASYMCHEM LABORATORIES (TIANJIN) CO.,LTD. The sequence listing filed with the application follows.

SEQUENCE LISTING (56 sequences)

SEQ ID NO: 1 - protein, 459 aa, Chromobacterium violaceum
MQKQRTTSQWRELDAAHHLHPFTDTASLNQAGARVMTRGEGVYLWDSEGNKIIDGMAGLWCVNVGYGRKDFAEAARRQMEELPFYNTFFKTTHPAVVELSSLLAEVTPAGFDRVFYTNSGSESVDTMIRMVRRYWDVQGKPEKKTLIGRWNGYHGSTIGGASLGGMKYMHEQGDLPIPGMAHIEQPWWYKHGKDMTPDEFGVVAARWLEEKILEIGADKVAAFVGEPIQGAGGVIVPPATYWPEIERICRKYDVLLVADEVICGFGRTGEWFGHQHFGFQPDLFTAAKGLSSGYLPIGAVFVGKRVAEGLIAGGDFNHGFTYSGHPVCAAVAHANVAALRDEGIVQRVKDDIGPYMQKRWRETFSRFEHVDDVRGVGMVQAFTLVKNKAKRELFPDFGEIGTLCRDIFFRNNLIMRACGDHIVSAPPLVMTRAEVDEMLAVAERCLEEFEQTLKARGLA

SEQ ID NO: 2 - protein, 459 aa, Chromobacterium violaceum
MQKQRTCSQWRELDAAHHLHPFTDTASLNQAGARVMTRGEGVYLWDCEGNKIIDGMAGLWCVNVGYGRKDFAEAARRQMEELPFYNTFYKTTHPAVVELSSLLAEVTPAGFDRVFYTNSGSESVDTMIRMVRRYWDVQGKPEKKTLIGRWNGYHGSTIGGASLGGFKAMHEQGDLPIPGMAHIEQPWWYKHGKDMTPDEFGVVAARWLEEKILEIGADKVAAFVGEPIQGAGGVIVPPATYWPEIERICRKYDVLLVADEVICGFGRTGEWFGHQHFGFQPDLFTAAKGLSSGYLPIGAVFVGKRVAEGLIAGGDFNHGFTYSGHPVCAAVAHANVAALRDEGIVQRVKDDIGPYMQKRWRETFSRFEHVDDVRGVGMALAFTLVKNKAKRELFPDFGEIGTLCRDIFFRNNLIMDSCGDHIVSAPPLVMTRAEVDEMLAVAERCLEEFEQTLKARGLA

SEQ ID NO: 3 - protein, 459 aa, Chromobacterium vaccinii
MQKQRTTSQWRELDAAHHLHPFTDTASLNQAGARVMTRGEGVYLWDSDGNKIIDGMAGLWCVNVGYGRKDFAEVARRQMEELPFYNTFFKTTHPAVVELSSLLAEVTPAGFDHVFYTNSGSESVDTMIRMVRRYWDVQGKPEKKTLIGRWNGYHGSTIGGASLGGMKYMHEQGDLPIPGMAHIEQPWWYKHGKDMTPDEFGVVAARWLDEKIQEIGADKVAAFVAEPIQGAGGVIIPPATYWPEIERICRKHDVLIVADEVICGFGRTGEWFGHQHFGFQPDLFTAAKGLSSGYLPIGAVFVGKRVAEGLIAGGDFNHGFTYSGHPVCAAVAHANVMALRDEGIVQRVKDDIGPYMQQRWRETFSQFEHVDDVRGVGLIQAFTLVKNKAKRELFPDFGEVGTLCRDIFFRNNLIMRACGDHIVCSPPLVMTRTEVDEMLGVAARCLAEFEQALKARGLA

SEQ ID NO: 4 - protein, 459 aa, Chromobacterium subtsugae
MQKQRTTSQWRELDAAHHLHPFTDTASLNQQGARVMTRGEGVYLWDSDGNKIIDGMAGLWCVNVGYGRHDFAEAARRQMEELPFYNTFFKTTHPAVVELSSLLAEVTPAGFERVFYTNSGSESVDTMIRMVRRYWDVKGKPQKKTLIGRWNGYHGSTIGGASLGGMKYMHEQGDLPIPGMAHIEQPWWYKHGKDMTPDEFGLVAARWLEEKILEIGADKVAAFVGEPIQGAGGVIIPPATYWPEIERICRKHDVLLVADEVICGFGRTGEWFGHQQLGFQPDIFTTAKGLSSGYLPIGAVFIGQRVAEGLIEGGDFNHGFTYSGHPVCAAVAHANVTALRDEGIVQRVKDDIGPYMQQRWRETFSRFEHVDDVRGVGLIQAFTLVKNKATRELFSDFGEVGTLCRDIFFRNNLIMRACGDHIVSAPPLVISRSEVDEMLAVASRCLEEFERTIKARGLV

SEQ ID NO: 5 - protein, 459 aa, Chromobacterium sphagni
MQKQRTTSQWRELDAAHHLHPFTDTASLNQQGARVMTRGEGVYLWDSEGNKIIDGMAGLWCVNVGYGRKDFAEVARRQMEELPFYNTFFKTTHPAVVELSSLLSEVTPAGFERVFYTNSGSESVDTMIRMVRRYWDVKGQPQKKTLIGRWNGYHGSTIGGASLGGMKYMHEQGDLPIPGMAHIEQPWWYKHGKDMTPEEFGLVAARWLEEKILEIGADKVAAFVGEPIQGAGGVIIPPASYWPEIERICRKYDVLIVADEVICGFGRTGEWFGHQGLGFTPDIFTAAKGLSSGYLPIGAVFIGQRVADGLIEGGDFNHGFTYSGHPVCAAVAHANVLALRDEGIVARVKDDIGPYMQKRWRETFSQFEHVDDVRGVGLIQAFTLVKNKATRELFPDFGEIGTLCRDIFFRNNLIMRACGDHIVSAPPLVISKAEVDEMLGVAARCLTEFEQTIKARGLV

SEQ ID NO: 6 - protein, 459 aa, unclassified Chromobacterium
MQKQRTTSQWRELDAAHHLHPFTDTASLNQAGARVMTRGEGVYLWDSDGNKIIDGMAGLWCVNVGYGRKDFADVARRQMEELPFYNTFFKTTHPAVVELSSLLAEVTPAGFDRVFYTNSGSESVDTMIRMVRRYWDVQGKPEKKTLIGRWNGYHGSTIGGASLGGMKYMHEQGDLPIPGMAHIEQPWWYKHGKDMTPDEFGLVAARWLEEKILEIGPDKVAAFVGEPIQGAGGVIIPPASYWPEIERICRKYDVLIVADEVICGFGRTGEWFGFQQLGFQPDIFTTAKGLSSGYLPIGAVFVGKRVAEGLIAGGDFNHGFTYSGHPVCAAVAHANVAALRDEGIVQRVKDDIGPYMQKRWRETFSQFEHVDDVRGVGMIQAFTLVKNKSKRELFADFGEIGTLCRDIFFRNNLIMRACGDHIVSAPPLVMTRAEVDAMLAVAARCLEEFEQTLKARGLA

SEQ ID NO: 7 - protein, 459 aa, Chromobacterium vaccinii
MQKQRTTSQWRELDAAHHLHPFTDTASLNQAGARVMTRGEGIYLWDSDGNKIIDGMAGLWCVNVGYGRKDFAEVARRQMEELPFYNTFFKTTHPAVVELSSLLAEVTPAGFEHVFYTNSGSESVDTMIRMVRRYWDVQGKPEKKTLIGRWNGYHGSTIGGASLGGMKYMHEQGDLPIPGMAHIEQPWWYKHGKDMTPDEFGVVAARWLDEKIQEIGADKVAAFVAEPIQGAGGVIIPPATYWPEIERICRKHDVLIVADEVICGFGRTGEWFGHQHFGFQPDLFTAAKGLSSGYLPIGAVFVGKRVAEGLVAGGDFNHGFTYSGHPVCAAVAHANVVALRDEGIVQRVKDDIGPYMQKRWRETFSQFEHVDDVRGVGLIQAFTLVKNKAKRELFPDFGEVGTLCRDIFFRNNLIMRACGDHIVCSPPLVMTRAEVDEMLGVAARCLAEFEQALKARGLA

SEQ ID NO: 8 - protein, 459 aa, Chromobacterium sp. 257-1
MQKQRSTSQWREMDAAHHLHPFTDTASLNQAGARVMTRGEGVYLWDSEGNKIMDGMAGLWCVNVGYGRKDFAEVARRQMEELPFYNTFFKTTHPAVIELSSLLSEVTPAGFDHVFYTNSGSESVDTMIRMVRRYWDVQGKPEKKTLIGRWNGYHGSTIGGASLGGMKYMHEQGDLPIPGMAHIEQPWWYKHGKDMTPDEFGLVAARWLEEKILEIGADKVAAFVGEPIQGAGGVIIPPATYWPEIERICRKHDVLLVADEVICGFGRTGEWFGHQQLGFQPDIFTTAKGLSSGYLPIGAVFVGKRVAEGLIAGGDFNHGFTYSGHPVCAAVAHANVVALRDEGIVRRVKEDIGPYMQQRWRETFSRFEHVDDVRGVGMIQAFTLVKNKATRELFPDFGEIGTLCRDIFFRNNLIMRACGDHIVSAPPLVMTRAEVDEMLALASRCLEEFEQALKARSLV

SEQ ID NO: 9 - protein, 459 aa, Chromobacterium sp. MWU14-2602
MQKQRTTSQWRELDAAHHLHPFTDTASLNEAGARVMTRGEGVYLWDSEGRKIMDGMAGLWCVNVGYGRKDFAEVARRQMEELPFYNTFFKTTHPAVVELSALLTEVTPAGFDHVFYTNSGSESVDTMIRMVRRYWDVQGKPQKKTLIGRWNGYHGSTIGGASLGGMKYMHEQGDLPIPGMAHIEQPWWYKHGKDMTPEEFGLVAARWLEEKILEIGADKVAAFVGEPIQGAGGVIIPPASYWPEIERICRKYDVLLVADEVICGFGRTGEWFGHQLFGFQPDIFTTAKGLSSGYLPIGAVFVGKRVAEGLIAGGDFNHGFTYSGHPVCAAVAHANVAALRDEGIVQRVKDDIGPYMQQRWRETFSRFEHVDDVRGVGMIQAFTLVKNKATRELFPDVGEAGTLCRDIFFRNDLIMRACGDHIVSAPPLVMTRAEVDEMLALAARCMEEFEQTLKARGLV

SEQ ID NO: 10 - protein, 459 aa, Chromobacterium sp. ATCC 53434
MQKQRTTSQWRELDAAHHLHPFTDTASLNQQGARVMTHGDGVYLWDSEGNKIIDGMAGLWCVNVGYGRKDFAEAARRQMDELPFYNTFFKTTHPAVVELSSLLAEVTPAGFDHVFYTNSGSESVDTMIRMVRRYWDVQGKPQKKTLIGRWNGYHGSTIGGASLGGMKYMHEQGDLPIPGMAHIEQPWWYKHGKDMTPEEFGVVAARWLEERILEIGADKVAAFVAEPIQGAGGVIIPPATYWPEIERICRKHDVLIVADEVICGFGRTGEWFGHQHFGFQPDLFTAAKGLSSGYLPIGAVFVGKRVAEGLAAGGDFNHGFTYSGHPVCAAVAHANVVALRDEGIVQRVKDDIGPYMQQRWRETFSRFEHVDDVRGVGMIQAFTLVKSKATRELFADFGDAGTLCRDIFFRNNLIMRACGDHIVSAPPLVMTRAEVDEMLTVAARCLEEFERTLKERGLV

SEQ ID NO: 11 - protein, 459 aa, Chromobacterium
MQNQRTTSQLRELDAAHHLHPFTDTASLNQAGARVMTRGEGVYLWDSEGNKIIDGMAGLWCVNVGYGRKDFAEVARRQMEELPFYNTFFKTTHPAVVELSALLCEVTPAGFDHVFYTNSGSESVDTMIRMVRRYWDVQGKPEKKTLIGRWNGYHGSTIGGASLGGMKYMHEQGDLPIPGMAHIEQPWWYKFGKDMTPDEFGLVAARWLEEKILEIGPEKVAAFVGEPIQGAGGVIIPPASYWPEIERICRKYDVLIVADEVICGFGRTGEWFGHQRLGFQPDIFTTAKGLSSGYLPIGAVFVGKRVAEGLIAGGDFNHGFTYSGHPVCAAVAHANVVALRDEGIVQRVKDDIGPYLQQRWRETFSRFEHVDDVRGVGMLGAFTLVKNKAKRELFPDFGEVGTLCRDIFFRNNLIMRACGDHIVSSPPLVMTRGEVDEMLAVAARCLEEFEQTIKARGLV

SEQ ID NO: 12 - protein, 459 aa, Xenophilus sp. AP218F
MQKQRTTSEWRELDAAHHLHPFTDTASLNHQGARIMTRGEGMYLWDSEGNKIIDGMAGLWCVNVGYGRKDFAEVARRQMEELPFYNTFFKTTHPAVVELSALLAEVTPAGFEHVFYTNSGSESVDTMIRMVRRYWDAQGKPEKKTLIGRWNGYHGSTIGGASLGGMKYMHEQGDLPIPGMAHVEQPWWYKHGKDMSRDEFGLAAARWLEEKILEIGADKVAAFVGEPIQGAGGVIIPPATYWPEVERICRKYDVLLVADEVICGFGRTGEWFGHQHFGFKPDMFTTAKGLSSGYLPMGAVFVGERVAKGLIAAGDFNHGFTYSGHPVCAAVARANVLALRDEGIVEQVKRDIGPYMQQRWRETFSQFKHVDDVRGVGLIQAFTLVKNKETRELFPNFGEVGLVCRDIFFRNNLIMRACGDHIVAAPPLVISKDDIDEMLAVAARCMREFEQKVESENLS

SEQ ID NO: 13 - protein, 460 aa, Chromobacterium sp. LK11
MQNQQRTTEQWRQLDAAHHLHPFTDTQSLNQQGARVMTRGEGIYLWDSEGNKIIDGMAGLWCVNVGYGRKELSDVAKHQMDELPFYNTFFKTTHPAVVELSHLLAQVTPAGYQHVFYTNSGSESVDTMIRMVRHYWDVQGKKDKKTLIGRWNGYHGSTIGGSSLGGMKYMHEQGDLPIAGMAHVEQPWWYKYGKDLSPDEFGVVAARWVEEKILEIGPEKVAAFVGEPIQGAGGVIIPPATYWPEVERICRKYDVLLVADEVICGFGRTGEWFGFEHFGFRPDIFTAAKGLSSGYLPIGAVFVGERVAQGLIAGGDFNHGFTYSGHPVASAVARANIELLRDEGIIDRVKNETGPYMQKRWRETFSQFEHVDDVRGVGLIQAFTLVKDKSKRELFPDFGDIGMMCRDIFFRNNLIMRACGDHIVASPPLVISKAEIDEMLGVAARCMEEFERKLKDDGLV

SEQ ID NO: 14 - protein, 460 aa, Chromobacterium sp. LK1
MQNQQRTTEQWRQLDASHHLHPFTDTQSLNQQGARVMTRGEGIYLWDSDGNKIIDGMAGLWCVNIGYGRKELSDVAKRQMDELAFYNTFFKTTHPAVVELSHLLAQVTPAGYEHVFYTNSGSESVDTMIRMVRHYWDVQGKKDKKTLIGRWNGYHGSTIGGSSLGGMKYMHEQGDLPIPGMAHVEQPWWYKYGKDLSPDEFGVVAARWVEEKILEIGPEKVAAFVGEPIQGAGGVIIPPATYWPEVERICRKYDVLLVADEVICGFGRTGEWFGFEHFGFRPDIFTTAKGLSSGYLPIGAVFVGERVAQGLIAGGDFNHGFTYSGHPVASAVARANVELLRDEGIIDRVKHETGPYMQQRWRETFSQFEHVDDVRGVGLIQAFTLVKDKSKRELFPNFGDVGLMCRDIFFRNNLIMRACGDHIVASPPLVITKAEIDEMLGVAARCMETFERKLKESGLA

SEQ ID NO: 15 - protein, 460 aa, Chromobacterium haemolyticum
MQNQQRTTEQWRQLDAAHHLHPFTDTQSLNQQGARVMTRSEGIYLWDSEGNKIIDGMAGLWCVNIGYGRKELSEVAKNQMDELPFYNTFFKTTHPAVVELSHLLAQVTPAGYEHVFYTNSGSEAVDTMIRMVRHYWDVQGKKDKKTLIGRWNGYHGSTIGGSSLGGMKYMHEQGDLPIPGMAHVEQPWWYKYGKDLSPDEFGVVAARWVEEKILEIGPEKVAAFVGEPIQGAGGVIIPPATYWPEVERICRKYDVLLVADEVICGFGRTGEWFGFEHFGFRPDIFTTAKGLSSGYLPIGAVFVGERVAQGLIAGGDFNHGFTYSGHPVASAVARVNIELLRDEGIIDRVKNETGPYMQKRWRETFSQFEHVDDVRGVGLIQAFTLVKDKSKRELFPEFGDVGLMCRDIFFSNNLIMRACGDHIVSAPPLVISKAEIDEMLGVAARCMETFERKLKDSGLV

SEQ ID NO: 16 - protein, 481 aa, Chromobacterium haemolyticum
MAKEGRQRTSTPRWRILEGSPMQNQQRTTEQWRQLDAAHHLHPFTDTQSLNQQGARVMTRSEGIYLWDSEGNKIIDGMAGLWCVNIGYGRKELSEVAKNQMDELPFYNTFFKTTHPAVVELSHLLAQVTPAGYEHVFYTNSGSEAVDTMIRMVRHYWDVQGKKDKKTLIGRWNGYHGSTIGGSSLGGMKYMHEQGDLPIPGMAHVEQPWWYKYGKDLSPDEFGVVAARWVEEKILEIGPEKVAAFVGEPIQGAGGVIIPPATYWPEVERICRKYDVLLVADEVICGFGRTGEWFGFEHFGFRPDIFTTAKGLSSGYLPIGAVFVGERVAQGLIAGGDFNHGFTYSGHPVASAVARVNIELLRDEGIIDRVKNETGPYMQKRWRETFSQFEHVDDVRGVGLIQAFTLVKDKSKRELFPEFGDVGLMCRDIFFSNNLIMRACGDHIVSAPPLVISKAEIDEMLGVAARCMETFERKLKDSGLV

SEQ ID NO: 17 - protein, 460 aa, Chromobacterium sp. Panama
MQNQQRTTEQWRQLDAAHHLHPFTDTQSLNQQGARVMTRSEGIYLWDSEGNKIIDGMAGLWCVNIGYGRKELSDVAKSQMDELPFYNTFFKTTHPAVVELSHLLAQVTPAGYEHVFYTNSGSEAVDTMIRMVRHYWDVQGKKEKKTLIGRWNGYHGSTIGGSSLGGMKYMHEQGDLPIPGMAHVEQPWWYKYGKDLSPDEFGVVAARWVEEKILEIGPEKVAAFVGEPIQGAGGVIIPPATYWPEVERICRKYDVLLVADEVICGFGRTGEWFGFEHFGFRPDIFTTAKGLSSGYLPIGAVFVGERVAQGLIAGGDFNHGFTYSGHPVASAVARVNIELLRDEGVIDRVKNETGPYMQKRWRETFSQFEHVDDVRGVGLIQAFTLVKDKSKRELFPEFGDVGLMCRDIFFSNNLIMRACGDHIVSAPPLVISKAEIDEMLGVAARCMETFERKLKDSGLV

SEQ ID NO: 18 - protein, 481 aa, Chromobacterium haemolyticum
MAKEGRQRTSTPRWRILEGSPMQNQQRTTEQWRQLDAAHHLHPFTDTQSLNQQGARVMTRSEGIYLWDSEGNKIIDGMAGLWCVNIGYGRKELSDVAKSQMDELPFYNTFFKTTHPAVVELSHLLAQVTPAGYEHVFYTNSGSEAVDTMIRMVRHYWDVQGKKDKKTLIGRWNGYHGSTIGGSSLGGMKYMHEQGDLPIPGMAHVEQPWWYKYGKDLSPDEFGVVAARWVEEKILEIGPEKVAAFVGEPIQGAGGVIIPPATYWPEVERICRKYDVLLVADEVICGFGRTGEWFGFEHFGFRPDIFTTAKGLSSGYLPIGAVFVGERVAQGLIAGGDFNHGFTYSGHPVASAVARVNIELLRDEGIIDRVKNETGPYMQKRWRETFSQFEHVDDVRGVGLIQAFTLVKDKSKRELFPEFGDVGLMCRDIFFSNNLIMRACGDHIVSAPPLVISKAEIDEMLGVAARCMETFERKLKDSGLV

SEQ ID NO: 19 - protein, 460 aa, Chromobacterium haemolyticum
MQNQQRTTEQWRQLDAAHHLHPFTDTQSLNQQGARVMTRSEGIYLWDSEGNKIIDGMAGLWCVNIGYGRKELSDVAKSQMDELPFYNTFFKTTHPAVVELSHLLAQVTPAGYEHVFYTNSGSEAVDTMIRMVRHYWDVQGKKDKKTLIGRWNGYHGSTIGGSSLGGMKYMHEQGDLPIPGMAHVEQPWWYKYGKDLSPDEFGVEAARWVEEKILEIGPEKVAAFVGEPIQGAGGVIIPPATYWPEVERICRKYDVLLVADEVICGFGRTGEWFGFEHFGFRPDIFTTAKGLSSGYLPIGAVFVGERVAQGLIAGGDFNHGFTYSGHPVASAVARVNIELLRDEGIIDRVKNETGPYMQKRWRETFSQFEHVDDVRGVGLIQAFTLVKDKSKRELFPEFGDVGLMCRDIFFSNNLIMRACGDHIVSAPPLVISKAEIDEMLGVAARCMETFERKLKDSGLV

SEQ ID NO: 20 - protein, 460 aa, Vogesella oryzae
MTQQQRSTAQWRELDAAHHLHPFTDTASLNEQGVRMITHADGIYLWDSEGNKITDGMAGLWCVNIGYGRKDLSEVAKRQMDELAYYNTFFKTSHPAVVELSHLLAEVAPAGFDHVFYTNSGSESVDTMIRMVRRYWDVKGKPQKKTLIGRWNGYHGSTIGGASLGGMSYMHEQGDLPIPGIAHIEQPWYYKHGKDMTPEEFGIAAAHWLEEKILEIGADKVAAFVGEPIQGAGGVIIPPSSYWPEVERICRKYDILLVADEVICGFGRTGEWFGHQHFGFKPDIFTTAKGLSSGYLPIGAVFVGNDVAATLAAGGDFNHGFTYSGHPVAAAVAHANVKALRDEGIVQRVKEETGPYMQQRWRETFGQFEHVDDVRGVGLIQAFTLVKNKATRELFDNWGEMGTMCRDIFFGNNLIMRACGDHIVSAPPLVITKAEIDATLATAARCIETFEKKLRERGLA

SEQ ID NO: 21 - protein, 459 aa, Vogesella urethralis
MTQQRNTAAWREMDAAHHLHPFTDTASLNEQGVRMITRADGIYLWDSEGNKIMDGMAGLWCVNIGYGRKDLSDVAKRQMDELAYYNTFFKTSHPAVVELSHLLAEVAPQGFDHVFYTNSGSESVDTMIRMVRRYWDVKGKPQKKTLIGRWNGYHGSTIGGASLGGMSYMHEQGDLPIPGIAHVEQPWYYKHGKDMTPEEFGVAAARWIEEKILEIGADKVAAFVGEPIQGAGGVIVPPSTYWPEVERICRKYDILLVADEVICGFGRTGEWFGHSHFGFTPDIYTTAKGLSSGYLPIGAVFVNDEVAATLAAGGDFNHGFTYSGHPVAAAVAHANVKALRDEGIVQRVKEDIGPYMQQRWRETFSQFEHVDDIRGVGLIQAFTLVKNKQTRELFDNWGEIGLMCRDIFFANNLIMRACGDHIVSAPPLVISKDEIDQMLATAARCMETFERKLKEKGLA

SEQ ID NO: 22 - protein, 460 aa, Vogesella sp. LIG4
MTQQQRSTAQWRELDAAHHLHPFTDTTSLNQQGVRMITHADGIYLWDSEGNKITDGMAGLWCVNLGYGRKDLSDVAKRQMDELAYYNTFFKTSHPAVVELSHLLAQVAPAGFDHVFYTNSGSESVDTMMRMVRRYWDVKGKPQKKTLIGRWNGYHGSTIGGASLGGMSYMHEQGDLPIPGIAHIEQPWYYKHGKDMTPEEFGLAAARWLEDKILEIGADKVAAFVGEPIQGAGGVIIPPSTYWPEVERICRKYDILLVADEVICGFGRTGEWFGQQHFGFKPDIFTTAKGLSSGYLPIGAVFVGNEVAATLAAGGDFNHGFTYSGHPVAAAVAHANVKALRDEGIVKRVKEETGPYMQQRWRETFGQFEHVDDVRGVGLIQAFTLVKNKATRELFDNWGEMGTMCRDIFFGNNLIMRACGDHMVSAPPLVITKAEIDTMLGTAARCMETFEQKLRERGLA

SEQ ID NO: 23 - protein, 459 aa, Aquitalea
MQNQRTTTEWRELDAAHHLHPFTDTNSLNQQGARVITKAEGIYLYDSEGNKILDGMAGLWCVNIGYGRKDLPEVAKQQMEQLAYYNTFFKTTHPAVVELSHLLSEVAPEGFKHVFYTNSGSESVDTMIRMVRRYWDVKGKKDKKTLIGRWNGYHGSTIGGASLGGMTYMHEQGDLPIPGIVHVEQPWWYKHGKDMTPEEFGLAAAKWVEDKILEVGADKVAAFVGEPIQGAGGVIVPPSTYWPEIQRICQKYDILLVADEVICGFGRTGEWFGQQVFGFKPDIFTTAKGLSSGYQPIGAVFVNDKVATTLAAGGDFNHGFTYSGHPVAAAVAHANVKALRDEGIVDRVKNDTGPYMQKRWREVFSQFEHVDDVRGVGLIQAFTLVKNKATRELFPDFGEIGTMCRDIFFKNNLIMRACGDHIVSAPPLVISKEEIDQMLETAAKCMVEFEKQLKERGLV

SEQ ID NO: 24 - protein, 459 aa, Aquitalea sp. LB_tupeE
MQNQRTTTEWRELDAAHHLHPFTDTNSLNQQGARVITKAEGIFLFDSEGNKILDGMAGLWCVNIGYGRKDLPEVAKQQMEQLAYYNTFFKTTHPAVVELSHLLSEVAPEGFKHVFYTNSGSESVDTMIRMVRRYWDVKGKKDKKTLIGRWNGYHGSTIGGASLGGMTYMHEQGDLPIPGIVHVEQPWWYKHGKDMTPEEFGLAAAKWVEDKILEVGADKVAAFVGEPIQGAGGVIVPPSTYWPEIQRICQKYDILLVADEVICGFGRTGEWFGQQVFGFKPDIFTTAKGLSSGYQPIGAVFVNDKVATTLAEGGDFNHGFTYSGHPVAAAVAHANVKALRDEGIVDRVKNDTGPYMQKRWREVFSQFEHVDDVRGVGLIQAFTLVKNKATRELFPDFGEIGTMCRDIFFKNNLIMRACGDHIVSAPPLVISKEEIDQMLETAAKCMVEFEQQLKARGLV

SEQ ID NO: 25 - protein, 459 aa, Vogesella perlucida
MTQQRNTAAWREMDAAHHLHPFTDTASLNEQGVRMITRADGIYLWDSEGNQIMDGMAGLWCVNIGYGRKDLSDVAKRQMDELAYYNTFFKTSHPAVVELSHLLADVAPQGFDHVFYTNSGSESVDTMIRMVRRYWDVKGKPEKKTLIGRWNGYHGSTIGGASLGGMSYMHEQGDLPIPGIVHVEQPWYYKHGKDMTQEEFGVAAARWIEEKILEVGADKIAAFVGEPIQGAGGVIVPPSTYWPEVQRICRQYDILLVADEVICGFGRTGEWFGQTHFGFQPDIFTTAKGLSSGYLPIGAVFVNDEVASTLAAGGDFNHGFTYSGHPVAAAVAHANVKALRDEGIVQRVKEDIGPYMQKRWRETFSQFEHVDDIRGVGLIQAFTLVKNKATRELFDNWGEIGLMCRDIFFANNLIMRACGDHIVSAPPLVISKAEVDQMIDTAARCMAEFERQLKEKGLA

SEQ ID NO: 26 - protein, 459 aa, Aquitalea
MQNQRTTTEWRELDAAHHLHPFTDTNSLNEQGARVITKADGIYLYDSEGNKILDGMAGLWCVNIGYGRKDLPEVAKRQMEQLAYYNTFFKTTHPAVVELSHLLAEVAPEGFKHVFYTNSGSESVDTMIRMVRRYWDVKGKKDKKTLIGRWNGYHGSTIGGASLGGMTYMHEQGDLPIPGIVHVEQPWWYKHGKDMTPEEFGLAAAKWVEDKILEVGADKVAAFVGEPIQGAGGVIVPPSTYWPEIQRICQKYDILLVADEVICGFGRTGEWFGQQVFGFKPDIFTTAKGLSSGYQPIGAVFVNDKVATTLAEGGDFNHGFTYSGHPVAAAVAHANVKALRDEGIVDRVKNDTGPYMQKRWREVFGQFEHVDDVRGVGLIQAFTLVKNKATRELFPNFGEIGTLCRDIFFKNNLIMRACGDHIVSAPPLVISKEEIDQMLDTAAKCMVEFEKQLKERGLA

SEQ ID NO: 27 - protein, 459 aa, Aquitalea denitrificans
MQNQRTTTEWRELDAAHHLHPFTDTNSLNQQGARVITKADGIYLYDSEGNKILDGMAGLWCVNIGYGRKDLPEVAKQQMEQLAYYNTFFKTTHPAVVELSHLLAEVAPEGFKQVFYTNSGSESVDTMIRMVRRYWDVKGKKDKKTLIGRWNGYHGSTIGGASLGGMTYMHEQGDLPIPGIVHVEQPWWYKHGKDMTPEEFGLAAAKWVEDKILEVGADKVAAFVGEPIQGAGGVIVPPSTYWPEIQRICQKYDILLVADEVICGFGRTGEWFGQQVFGFKPDIFTTAKGLSSGYQPIGAVFVNEKVATTLAEGGDFNHGFTYSGHPVAAAVAHANVKALRDEGIVDRVKNDTGPYMQKRWREVFGQFEHVDDVRGVGLIQAFTLVKNKATRELFPNFGEIGTMCRDIFFKNNLIMRACGDHIVSAPPLVISKEEIDQMLETAAKCMVEFEKQLKERGLV

SEQ ID NO: 28 - protein, 459 aa, Aquitalea
MQNQRTTTEWRELDAAHHLHPFTDTNSLNQQGARVITKAEGIFLYDSEGNKILDGMAGLWCVNIGYGRKDLPEVAKQQMEQLAYYNTFFKTTHPAVVELSHLLSEVAPEGFKHVFYTNSGSESVDTMIRMVRRYWDVKGKKDKKTLIGRWNGYHGSTIGGASLGGMTYMHEQGDLPIPGIVHVEQPWWYKHGKDMTPEEFGLAAAKWVEDKILEVGADKVAAFVGEPIQGAGGVIVPPSTYWPEIQRICQKYDILLVADEVICGFGRTGEWFGQQVFGFKPDIFTTAKGLSSGYQPIGAVFVNEKVATTLAEGGDFNHGFTYSGHPVAAAVAHANVKALRDEGIVDRVKNDTGPYMQKRWREVFGQFEHVDDVRGVGLIQAFTLVKNKATRELFPNFGEIGTMCRDIFFKNNLIMRACGDHIVSAPPLVISKEEIDQMLETAAKCMVEFEQQLKERGLV

SEQ ID NO: 29 - protein, 459 aa, Aquitalea sp. FJL05
MQNQRTTTEWRELDAAHHLHPFTDTNSLNEQGARVITKADGIYLYDSEGNKILDGMAGLWCVNIGYGRKDLPEVAKRQMEQLAYYNTFFKTTHPAVVELSHLLAEVAPEGFKHVFYTNSGSESVDTMIRMVRRYWDVKGKKDKKTLIGRWNGYHGSTIGGASLGGMTYMHEQGDLPIPGIVHVEQPWWYKHGKDMTPEEFGLAAAKWVEDKVLEVGADKVAAFVGEPIQGAGGVIVPPSTYWPEIQRICQKYDILLVADEVICGFGRTGEWFGQQVFGFTPDIFTTAKGLSSGYQPIGAVFVNEKVATTLAEGGDFNHGFTYSGHPVAAAVAHANVKALRDEGIVDRVKNDTGPYMQKRWREVFGQFEHVDDVRGVGLIQAFTLVKNKATRELFPNFGEIGTLCRDIFFKHNLIMRACGDHIVSAPPLVISKEEIDQMLDTAAKCMVEFEKQLKERGLA

SEQ ID NO: 30 - protein, 421 aa, Aquitalea magnusonii
MDGIYLYDSEGNKILDGMAGLWCVNIGYGRKDLPEVAKRQMEQLAYYNTFFKTTHPAVVELSHLLAEVAPQGFKHVFYTNSGSESVDTMIRMVRRYWDVKGKKDKKTLIGRWNGYHGSTIGGASLGGMTYMHEQGDLPIPGIVHVEQPWWYKHGKDMTPEEFGLAAAKWVEDKILEVGADKVAAFVGEPIQGAGGVIVPPSTYWPEIQRICQKYDILLVADEVICGFGRTGEWFGQQVFGFTPDIFTTAKGLSSGYQPIGAVFLNDKVATTLAEGGDFNHGFTYSGHPVAAAVAHANVKALRDEGIVDRVKNDTGPYMQKRWREVFGQFEHVDDVRGVGLIQAFTLVKNKATRELFPNFGEIGTLCRDIFFKNNLIMRACGDHIVSAPPLVISKEEIDQMLETAAKCMVEFEKQLKERGLV

SEQ ID NO: 31 - protein, 459 aa, Pseudogulbenkiania sp. MAI-1
MQNERTTAQWRALDAAHHLHPFTDTESLNQQGARVITKADGVFLWDSEGNKILDGMAGLWCVNIGYGRKDLSEVAKRQMDELAYYNTFFKTTHPAVVELSRLLSEVAPQGFSRIFYTNSGSESVDTMIRMVRRYWDVKGKPEKKTLIGRWNGYHGSTIGGASLGGMSYMHEQGDLPIPGITHVEQPWWYRYGQGMTPEEFGVVAARWVEEKILEVGPDKVAAFVGEPIQGAGGVIIPPSTYWPEVERICRQYDVLLVADEVICGFGRTGEWFGHQLFGFRPDLFTAAKGLSSGYLPIGAVFVGDKVAQGLIEGGDFNHGFTYSGHPVAAAVAHANVKALRDEGIIDRVKHDTGPYMQQRWRAAFGGFAHVDDVRGVGLIQAFTLVKDKATHELFPDWGTVGTICRDIFFRHNLIMRACGDHMVAAPPLVISKAEIDQLIETAVQCVTECEQVLRERGLV

SEQ ID NO: 32 - protein, 459 aa, Paludibacterium paludis
MSQQRTTAEWRALDAAHHVHPFSDAHSLNRQGARVMTRADGIYLWDSDGNKIIDGMAGLWCVNIGYGRHDMTAAASRQMDELPFYNTFFKTTHPAVVELSALLAKVAPEGFNHVFYTNSGSESVDTMIRMVRRYWDVAGKPSKKTLIGRWNGYHGSTMGGASLGGMDYMHAQGGLPIPDMAHIEQPWWYKFGKDMSRDEFGLLAAGWLEDRILEIGPDNVAAFVGEPIQGAGGVIIPPDTYWPEIERICRKYDVLLVADEVICGFGRTGEWFGQQRFGFRPDIFTAAKGLTSGYLPMGAVFLNEKVAEGLAAGGDFNHGFTYSGHPVAAAVARANILALRDEGIIDRVRHDTGPYMQERWRQVFGQFDHVDDVRGVGLIQAFTLVKDKATRTLFPNWGETGLICRDIFFRNNLIMRACADHMVASPPLVMTRAQIDEMLGVAERCMTEFEETLLRRGLV

SEQ ID NO: 33 - protein, 459 aa, Pseudogulbenkiania sp. NH8B
MQSERTTEQWRALDAAHHLHPFTDTESLNQQGARVITKADGVFLWDSDGNKILDGMAGLWCVNIGYGRKDLSEVARRQMDELAYYNTFFKTTHPAVVELSHLLSQVAPEGFSRIFYTNSGSESVDTMIRMVRRYWDVKGRPGKKTLIGRWNGYHGSTIGGASLGGMSYMHEQGDLPIPGIVHVEQPWWYRYGQGMSPEEFGVVAARWVEEKILEVGPDKVAAFVGEPIQGAGGVIIPPSTYWPEVERICRRYDVLLVADEVICGFGRTGEWFGHQLFGFKPDLFTAAKGLSSGYLPIGAVFVGDKVAQGLAEGGDFNHGFTYSGHPVAAAVAHANVKALRDEGIIDRVKHDTGPYMQQRWREAFGGFAHVDDVRGVGLIQAFTLVKDKATHELFPNWGEVGTICRDIFFRHNLIMRACGDHMVAAPPLVISKTEIDQLIDTAVQCVTECEAVLRQRGLV

SEQ ID NO: 34 - protein, 459 aa, Pseudogulbenkiania subflava
MQNERTTEQWRALDAAHHLHPFTDTESLNQQGARVITKADGVFLWDSDGNKILDGMAGLWCVNIGYGRKDLSEVAKRQMDELAYYNTFFKTTHPAVVELSQLLSEVAPKGFSRIFYTNSGSESVDTMIRMVRRYWDVKGKPGKKTLIGRWNGYHGSTIGGASLGGMSYMHEQGDLPIPGIEHVEQPWWYRYCQGMSPEEFGVVAARWLEAKILEIGPDKVAAFVGEPIQGAGGVIIPPSTYWPEVERICRQYDVLLVADEVICGFGRTGEWFGHQLFGFHPDLFTAAKGLSSGYLPIGAVFVGDKVAQGLAEGGDFNHGFTYSGHPVAAAVAHANVKALRDEGIIDRVKRDTGPYMQQRWREAFGGFAHVDDVRGVGLIQAFTLVKDKATHELFPNWGEVGTICRDIFFRHNLIMRACGDHMVAAPPLVISKAEIDQLIDTAVQCVTECEEVLRQRGLV

SEQ ID NO: 35 - protein, 459 aa, Pseudogulbenkiania ferrooxidans
MQSERTTEQWRALDAAHHLHPFTDTESLNQQGARVITKADGVFLWDSDGNKILDGMAGLWCVNIGYGRKDLSEVARRQMDELAYYNTFFKTTHPAVVELSHLLSQVAPEGFSHIFYTNSGSESVDTMIRMVRRYWDVKGKPGKKTLIGRWNGYHGSTIGGASLGGMSYMHEQGDLPIPGIVHVEQPWWYRYGQGMSPEEFGVVAARWVEEKILEVGPDKVAAFVGEPIQGAGGVIIPPSTYWPEVERICRRYDVLLVADEVICGFGRTGEWFGHQLFGFHPDLFTAAKGLSSGYLPIGAVFVGDKVAQGLAEGGDFNHGFTYSGHPVAAAVAHANVKALRDEGIIDRVKHDTGPYMQQRWREAFGGFAHVDDVRGVGLIQAFTLVKDKATHELFPNWGEVGTICRDIFFRHNLIMRACGDHMVAAPPLVISKAEIDQLIDTAVQCVTECEAVLHQRGLV

SEQ ID NO: 36 - protein, 460 aa, Gulbenkiania indica
MQTARTTEQWRELDAAHHLHPFTDPHSLNQQGARVITRGEGIHLWDSEGHKIIDGMAGLWCVNIGYGRKDLPEVARRQMEDLAYYNTFFKTTHPAVVELSHLLSEVAPEGFRHIFYTNSGSESVDTMMRMVRHFWAVQGKPEKKVLIGRWNGYHGSTIGGASLGGMTYMHEQGDLPIPGIEHVEQPWWYKYGKDMTPEEFGLAAARWVEDKILEVGPERVAAFVGEPIQGAGGVIIPPSTYWPEVERICRKYDVLLVADEVICGFGRTGEWFGQQTMGFHPDIFTTAKGLSSGYLPIGAVFVGDRVANVLVAGGDFNHGFTYSGHPVAAAVAHANVKALRDEGIVDRVKNETGPYMQERWRATFGNFDHVDDVRGVGLIQGFTLVRNKATHELFPEWGTAGTMCRDIFFENNLIMRACGDHIVAAPPLVITKAEIDEMLGVAGRCLERFEKVVREKGMAG

SEQ ID NO: 37 - protein, 459 aa, Paludibacterium sp. dN 18-1
QKQRSTRELRELDAAHHLHPFTDTTSLNQQGARVITKGEGIYLWDSEGNKIIDGMAGLWCVNIGYGRKDLSEVAKRQMDDLAYYNTFFKTTHPAVVELSHLLAEVAPAGFSHVFYTNSGSESVDTMIRMVRRYWEVKGQKQKKTLIGRWNGYHGSTIGGASLGGMAYMHQDGGDLPIPGIEHVQQPWWYGLGGDMTPEEFGLAAAKWLEDKILEIGPDKVAAFVGEPIQGAGGVIIPPSTYWPEVERICHKYDVLLVADEVICGFGRTGEWFGHQCFGFHPDIFTTAKGLSSGYLPIGAVFVGDKVAAMLAEGGDFNHGFTYSGHPVAAAVACANVRALRDEGIIERVKHETGPYMQQRWREVFSRFEHVGDVRGVGLIQAFTLVKNKATRELFPNTGEIGLICRDIFFRHDLIMRACGDHMVSAPPLVISKQEIDDMLALAAQCMEEFEAELKARNLV

SEQ ID NO: 38 - protein, 459 aa, Vogesella fluminis
MKHQRSTAQWREMDAAHHLHPFTDTASLNAQGVRMITHADGIYLWDSEGNKIIDGMAGLWCVNIGYGRKDLPEIAKRQMEELAYYNTFFKTSHPAVVELSHLLAEVAPKGFDHVFYTNSGSESVDTMIRMVRRYWDVKGKPQKKTLIGRWNGYHGSTIGGASLGGMSYMHEQGDLPIPGIVHVQQPWHYKYGKGMSADEFGLLAASWIEDKILEVGADKVAAFVGEPIQGAGGVIIPPASYWPEVERICRKYDILLVADEVICGFGRTGHWFGQQQFGFTPDIFTTAKGLSSGYLPIGAVFVGNEVAATLAAGGDFNHGFTYSGHPVAAAVAHANVKALRDEGIVAAVHEDTGPYMQKRWREAFSRFEHVDDVRGVGLIQAFTLVKDKASQTLFDNWGEIGLMCRDIFFRHGLIMRACGDHIVSAPPLIISKDQIDEMIATAVECMEIFEQKLKERGLA

SEQ ID NO: 39 - protein, 459 aa, Vogesella alkaliphila
MKHQRSTAQWREMDAAHHLHPFTDTASLNEQGVRMITHADGIYLWDSEGNKILDGMAGLWCVNIGYGRKDLPEVAKRQMEELAYYNTFFKTSHPAVVELSHLLAEVAPKGFDHVFYTNSGSESVDTMIRMVRRYWDVKGKPEKKTLIGRWNGYHGSTIGGASLGGMSYMHEQGDLPIPGIVHVQQPWHYKYGKGMSADEFGKLAASWVEDKILEVGADKVAAFVGEPIQGAGGVIIPPATYWPEVERICRKYDILLVADEVICGFGRTGHWFGHQQFGFTPDIFTTAKGLSSGYMPIGAVFVNNEVAATLAAGGDFNHGFTYSGHPVAAAVAHANVKALRDEGIVAAVHEDTGPYMQKRWREAFSRFEHVDDVRGVGLIQAFTLVKDKASQTLFDNWGEIGLMCRDIFFKHGLIMRACGDHIVSAPPLIISKDQIDELIATAVKCMEIFEQQLKERGLA

SEQ ID NO: 40 - protein, 458 aa, Crenobacter sp. HX-7-9
MKQNTEAWRALDAAHHLHPFSDTKGLNAQGARVITRAEGIYLWDSEGNQIIDGMAGLWCVNIGYGRKDLAEVAKRQMEELAYYNTFFKTTNPQVAELSKLLAEVAPEGFEHVFYTNSGSESVDTMIRMVRHYWSSVGKPEKKVLIGRWNGYHGSTIGGASMGGMTYMHEQGDLPIPGIVHVEQPWYYKHGKDMTPEEFGLAAARWIEDKILEVGADKVAAFVGEPIQGAGGVIIPPATYWPEVERICRKYDILMVCDEVICGFGRTGQWFGHELYGVKPDLFTTAKGLSSGYLPIGAVFVGERVAQGLIEHGGDFNHGFTYSGHPVCCAVARANVTALRDEGIVARVREETGPYMQAKWRETFGQFDHVDDVRGVGLIQAFTLVKDKQKRELFDNWGTMGLACRDIFFRENLIMRACGDHIVAAPPLVISKREIDEMLGRAARCVEEFERVVVRGQPG

SEQ ID NO: 41 - protein, 459 aa, Vogesella indigofera
MKHQRSTAQWREMDAAHHLHPFTDTASLNEQGVRMITHADGIYLWDSEGNKILDGMAGLWCVNIGYGRKDLPEVAKRQMEELAYYNTFFKTSHPAVVELSHLLAEVAPKGFDHVFYTNSGSESVDTMIRMVRRYWDVKGKPEKKTLIGRWNGYHGSTIGGASLGGMSYMHEQGDLPIPGIVHVQQPWHYKYGKGMSADEFGKLAASWIEDKILEVGADKVAAFVGEPIQGAGGVIIPPASYWPEVERICRKYDILLVADEVICGFGRTGHWFGQQQFGFTPDIFTTAKGLSSGYMPIGAVFVNNEVATTLAAGGDFNHGFTYSGHPVAAAVAHANVKALRDEGIVAAVHEDTGPYMQKRWREAFSRFEHVDDVRGVGLIQAFTLVKDKASQTLFDNWGEIGLMCRDIFFKHGLIMRACGDHIVSAPPLIISKDQIDELITTAVKCMEIFEQQLKERGLA

SEQ ID NO: 42 - protein, 458 aa, Crenobacter sp. GY 70310
MKQNTEAWRALDAAHHLHPFSDTKGLNAQGARVITRAEGIYLWDSEGNQIIDGMAGLWCVNIGYGRKDLAEVAKRQMEELAYYNTFFKTTNPQVAELSKLLAEVAPDGFEHVFYTNSGSESVDTMIRMVRHYWSSVGKPEKKVLIGRWNGYHGSTIGGASMGGMTYMHEQGDLPIPGIVHVEQPWYYKHGKDMTPEEFGLAAARWIEDKILEVGADKVAAFVGEPIQGAGGVIIPPATYWPEVERICRKHDILMVCDEVICGFGRTGQWFGHELYGVKPDLFTTAKGLSSGYLPIGAVFVGERVAQGLIEHGGDFNHGFTYSGHPVCCAVARANVTALRDEGIVARVREETGPYMQAKWRETFGQFEHIDDVRGVGLIQAFTLVKDKQKRALFDNWGTMGLACRDIFFRENLIMRACGDHIVAAPPLVISKPEIDEMLGRAARCVEEFERVVVRGQPG

SEQ ID NO: 43 - protein, 459 aa, Vogesella sp. EB
MKHQRSTAQWREMDAAHHLHPFTDTASLNGQGVRMITHADGIYLWDSEGNKILDGMAGLWCVNIGYGRKDLPEVAKRQMEELAYYNTFFKTSHPAVVELSHLLAEVAPKGFDHVFYTNSGSESVDTMIRMVRRYWDVKGKPQKKTLIGRWNGYHGSTIGGASLGGMSYMHEQGDLPIPGIVHVQQPWHYKYGKGMSADEFGKLAASWIEDKILEVGADKVAAFVGEPIQGAGGVIIPPASYWPEVERICRKYDILLVADEVICGFGRTGHWFGQQQLGFTPDIFTTAKGLSSGYMPIGAVFVNNEVAATLAAGGDFNHGFTYSGHPVAAAVAHANVKALRDEGIVAAVHEDTGPYMQKRWREAFSRFEHVDDVRGVGLIQAFTLVKDKASQTLFDNWGEIGLMCRDIFFKHGLIMRACGDHIVSAPPLIISKDQIDELITTAVKCMEIFEQQLKERGLA

SEQ ID NO: 44 - protein, 457 aa, Rhodobacteraceae bacterium CH30
SQQHTTQDWRAMDAAHHLHPFSDTKGLNAQGARVITHADGIYLWDSEGNKITDGMAGLWCVNIGYGRKDLPEVAKRQMEELAYYNTFFKTTHPKVAELSALLASVAPDGFEHVFYTNSGSESVDTMIRMVRHYWSSVGKPEKKVLIGRWNGYHGSTIGGASLGGMSYMHEQGDLPIPGIAHVEQPWYYKHGKDLTPEEFGIQAAQWIEAKILEVGADKVAAFVGEPVQGAGGVIIPPSTYWPEVERICRKYDVLLVADEVICGFGRTGEWFGQTHFGFKPDMFTTAKGLSSGYLPIGAVFVGERVARGLIEEGGDFNHGFTYSGHPVCAAVAHANVAALRDEGIVERVKNETGPYMQQRWREVFGQFAHVDDVRGVGLIQAFTLVKNKATRELFDNWGEAGTQCRDIFFKHNLIMRACGDHIVCAPPLVITKAEIDAMLETAVACLREFEQLVAARS

SEQ ID NO: 45 - protein, 458 aa, Neisseriaceae bacterium B2N2-7
MSQQHTTQDWRAMDAAHHLHPFSDTKGLNAQGARVITHADGIYLWDSEGNKITDGMAGLWCVNIGYGRKDLPEVAKRQMEELAYYNTFFKTTHPKVAELSALLASVAPDGFEHVFYTNSGSESVDTMIRMVRHYWSSVGKPEKKVLIGRWNGYHGSTIGGASLGGMSYMHEQGDLPIPGIAHVEQPWYYKHGKDLTPEEFGIQAAQWIEAKILEVGADKVAAFVGEPVQGAGGVIIPPSTYWPEVERICRKYDVLLVADEVICGFGRTGEWFGQTHFGFKPDMFTTAKGLSSGYLPIGAVFVGERVARGLIEEGGDFNHGFTYSGHPVCAAVAHANVAALRDEGIVERVKNATGPYMQQRWREVFGQFAHVDDVRGVGLIQAFTLVKNKATRELFDNWGEAGTQCRDIFFKHNLIMRACGDHIVCAPPLVITKAEIDAMLETAVACLREFEQLVAARS

SEQ ID NO: 46 - protein, 461 aa, Microvirgula
MSTTARSTNEYRELDAAHHLHPFSDMGSLNRQGSRVIVKGDGIYLWDSEGNKITDGMAGLWCVNIGYGRKDLAEVARQQMEDLAYYNTFFKTTHPRVVELSTLLAEVTQPGYQHVFYTNSGSESVDTVIRMVRQYWSIKGKPGKKTLISRWNGYHGSTIGGASLGGMTYMHEQGDLPIPGIAHIGQPWYLKEGRDGESEADFGLRAASWLEEKILEIGADKVAAFVGEPILGAGGVIIPPASYWPEIERICNKYDILLVADEVICGFGRTGDWFGHEHFGFRPHLFTIAKGLSSGYLPIGGVIIGDEVARTLIEGGDFNHGFTYSGHPVSAAVAHANVRALRDEGIVEQVKKDTGPYMQKRWREAFGGFEHVTDVRGVGLIQAFTWVKNKATREMFAGSDDVGTLCRDIFFKHNLIMRACGDSMVSAPPLIITRTEIDAMLSTAVECVEQTEKLLQERGLV

SEQ ID NO: 47 - protein, 469 aa, Neisseria shayeganii
MSKQDYSRQDGKHHLHPFSDNAALAREGVRVMVKAKGIYVYDDEGNEILDGMAGLWCVNIGYGRKELAKVAKKQMKELPFYNTFFKTTHPAVVELSSTITDIAPSGFNHVFYTGSGSESVDTMMRMVRHYWASVGKPQKKVIIGRWNGYHGSTIGGASLGGMKGMHNQGDLPIPNVVHIEQPWYYGLAKDGETPEEFGLRAANWLEEKIEEIGADKIAAFVGEPIQGAGGVIIPPKTYWPRIEEICRKHDILLVADEVICGFGRTGNWFGHETMGFKPDIFTTAKGLSSGYLPIGAVLVNDKVAEGLKAGGEFNHGFTYSGHPVAAAVAKKNLEILQDEGIVDQVKNETGPYMKKRWEETFSQFKYVDDIRSEGLICGFTLVKDKATRELFPNTGETGLMCRDIFFKNNLIMRACGDHMVAAPPLVMTKKEIDKMLAVAEQCMREFEQMMDKKLAKEEKAGKKEEKSDQ

SEQ ID NO: 48 - protein, 469 aa, Neisseria shayeganii
MSKQDYSRQDGKHHLHPFSDNAALAREGVRVMVKAKGIYVYDDEGNEILDGMAGLWCVNIGYGRKELAKVAKKQMKELPFYNTFFKTTHPAVVELSATITDIAPSGFNHVFYTGSGSESVDTMMRMVRHYWASVGKPQKKVIIGRWNGYHGSTIGGASLGGMKGMHSQGDLPIPNVVHIEQPWYYGLAKDGESPEEFGLRAANWLEEKIEEIGADKIAAFVGEPIQGAGGVIIPPKTYWPRIEEICRKHDILLVADEVICGFGRTGNWFGHETMGFKPDIFTTAKGLSSGYLPIGAVLVNDKVAEGLKAGGEFNHGFTYSGHPVAAAVAKKNLEILQDEGIVDQVKNETGPYMKKRWEETFSQFKYVDDIRSEGLICGFTLVKDKARRELFPNTGETGLMCRDIFFKNNLIMRACGDHMVAAPPLVMTKKEIDKMLAVAEQCMREFEQMMDKKLAKEEKAGKKEEKSDQ

SEQ ID NO: 49 - protein, 478 aa, Vitreoscilla sp. C1
MYKKSTIRIFATTSHKMNIDKEINMTNTTLNATANHLHPFSDNQQLKEKGVRVITKADGIYIYDDAGNKIIDGMAGLWCVNIGYGRKELADIARDQMNELAYYNTFFKTSHPAVINLSAKLASIAPAGFNHVFYTGSGSESVDSMIRMVRHYWDSVGKPSKKTLIGRWNGYHGSTIGGVSMGGMKGMHKQGGFPIEGIVHIEQPWFYGLHEEGETAEQFGIRAANWLEEKILEIGADNVAAFVGEPIQGAGGVIIPPSTYWPRIQEICQKYDILLVADEVICGFGRTGEWFGHETFGFQPDIFTTAKGLSSGYLPIGAVFVGDKVVEGILKGGDFNHGFTYAGHPVAAAVALKNVEILDDEGIIKNVHDKTGPYMQAKWREMLSQFKYVDDVRGVGLIQGFTLVKNKATREMFPNEGETGTMLRDIFFSNNLIMRACGDHIVASPPLTITKEEIDLMLATAEKCLQEFETAMDSKLGA

SEQ ID NO: 50 - protein, 454 aa, Vitreoscilla
MTNTTLNATANHLHPFSDNQQLKEKGVRVITKADGIYIYDDAGNKIIDGMAGLWCVNIGYGRKELADIARDQMNELAYYNTFFKTSHPAVINLSAKLASIAPAGFNHVFYTGSGSESVDSMIRMVRHYWDSVGKPSKKTLIGRWNGYHGSTIGGVSMGGMKGMHKQGGFPIEGIVHIEQPWFYGLHEEGETAEQFGIRAANWLEEKILEIGADNVAAFVGEPIQGAGGVIIPPSTYWPRIQEICQKYDILLVADEVICGFGRTGEWFGHETFGFQPDIFTTAKGLSSGYLPIGAVFVGDKVVEGILKGGDFNHGFTYAGHPVAAAVALKNVEILDDEGIIKNVHDKTGPYMQAKWREMLSQFKYVDDVRGVGLIQGFTLVKNKATREMFPNEGETGTMLRDIFFSNNLIMRACGDHIVASPPLTITKEEIDLMLATAEKCLQEFETAMDSKLGA

SEQ ID NO: 51 - protein, 462 aa, Laribacter hongkongensis
MTADPRRTEHYRELDAAHHLHPFSDMEALNRQGSRVMVRGEGIHVWDSDGVRLIDGMAGLWCVNLGYGRRDLAEAAYAQLCELPYYNTFFKTTHPRVAELSALVAEVAPPGFSHVFYTNSGSEAVDTMMRMVRHYWALKGQPQKKVLIGRWNGYHGSTLGGASLGGMPAMHAQGDLPVADVVHVEQPWFLKHGLDGETEEAFGLRAARWVEEKILETGADRVAAFVGEPIQGAGGVIIPPASYWPEVERICRRHDVLLVADEVICGFGRTGEWFGHQLYGIRPDLFTVAKGLSSGYLPIGGVVVGDEVAQVIKAGGDFNHGFTYSGHPACAAVAAANVRALRDEGVVERVRQDTGPYMQQRWREAFGGFAHLADIRGVGLIQGFTWVQDKELRRLFPDWGEVGLLCRDVFFRHNLIMRACGDHMVAAPPLVINRDEVDAMLEVAVQCVAETESVLRERGLID

SEQ ID NO: 52 - protein, 462 aa, Laribacter hongkongensis
MTADPRRTEHYRELDAAHHLHPFSDMEALNRQGSRVMVRGEGIHVWDSDGVRLIDGMAGLWCVNLGYGRRDLAEAAYAQLCELPYYNTFFKTTHPRVAELSALVAEVAPPGFHHVFYTNSGSEAVDTMMRMVRHYWALKGQPQKKVLIGRWNGYHGSTLGGASLGGMPAMHAQGDLPVADVVHVEQPWFLKHGLDGETEEAFGLRAARWVEEKILETGADRVAAFVGEPIQGAGGVIIPPASYWPEVERICRRHDVLLVADEVICGFGRTGEWFGHQLYGIRPDLFTVAKGLSSGYLPIGGVVVGDAVAQVIKAGGDFNHGFTYSGHPACAAVAAANVRALRDEGVVERVRQDTGPYMQQRWREAFGGFAHLADIRGVGLIQGFTWVQDKELRRLFPDWGEVGLLCRDVFFRHNLIMRACGDHMVAAPPLVINRDEVDAMLEVAVQCVAETESVLRERGLID

SEQ ID NO: 53 - protein, 462 aa, Rivicola pingtungensis; identical to SEQ ID NO: 52

SEQ ID NO: 54 - protein, 460 aa, Stenoxybacter acetivorans
MSKKNYSKHDVKHHLHPFSDNAALQEEGVRVMVKAKGVYVYDNDGNEILDGMAGLWCVNVGYGRKELVRAAKKQMEILPFYNTFFKTTHPAAVELTDKLVEITPEGFNHVFYTGSGSESVDTMMRMVRHYWASIGKPEKKIIIGRWNGYHGSTIGGASLGGMKGMHEQGDLPIPNVVHIEQPWYYGLAKDNETAGEFGIRAANWLEEKITELGADKVAAFVGEPIQGAGGVIVPPDGYWQRIEEICRKHDILLVADEVICGYGRTGNWFGHETFGFKPDIFTTAKGLSSGYIPIGAVLVNDRVTEGLLAGGEFNHGFTYSGHPVAAAVARANLDILDNEEIVDRIHDKIGPYMKKRWQETFEPFKYVGDIRSVGLMCGFTLVKNKETREFFPNTGETGLICRDIFFKNNLIMRACGDHIVAAPPLVISKKEIDHMLSIAAKCMREFEVKMDQILAKQDQD

SEQ ID NO: 55 - protein, 461 aa, Aquaspirillum sp. LM1
MTLATRSTADWQALDAAHHLHPFSDTQSLNQTGSRVVVKGDGVYIWDSEGNRIIDGMAGLWCVNLGYGREELADAAYQQMRELPFYNTFFKTTHPPVIELSALLAELTPPQFNHVFLTNSGSEANDTVIRMVRHFWAAQGQASKKVLIGRWNGYHGSTIGGASLGGMRYMHEQGDLPIPGIEHIEQPYWYVNGGELSPHDYGLKAAQALEAKILALGADNVAAFVGEPIQGAGGVIVPPDSYWPEIQRICRAYNILLVVDEVICGFGRTGQWFGSQHFGIEPDLMPIAKGLSSGYQPIGGVMVSDRVAQVLIQEGGDFNHGMTYSGHPVAAAVAVANLKILRDEGIVDQVREKTGPYLQQKWRETFAGHPYLDDVRGVGFLAAFTWVKDKSRRELFAEPGTVGTICRDIFFKNNIIMRAVGDSMVCAPPLVMTTTEIDEMIALAARCVDLTVQALEARGLV

SEQ ID NO: 56 - protein, 459 aa, Paludibacterium yongneupense
MAQERSTQQWRDMDAAHHLHPFTDTDSLNRHGARVITHGEGIYLWDSDGNKITDAMAGLWCVNLGYGRKDLALVAQQQMETLAYYNTFFKTTHPAVTELSALLSEIAPPGFSRMFYTNSGSEAVDTMIRMVRRYWDVQGQPQKKTLIGRWNGYHGSTIGGASLGGMGYMHEQGDLPIPGIAHIEQPWWYGLGGDSSREAFGLHAAGWLEQKILEIGADKVAAFVGEPIQGAGGVIIPPASYWPEIERICRKYDVLLVADEVICGFGRTGEWFGHQHFGFHPDLFTTAKGLSSGYQPIGAVFVGDRVAEGLARGGDFNHGFTYSGHPVAAAVARATVRALRDDGIVDRVKNDVGPYMQERWRETFEGFDHVDDVRGVGLIQGFTLVRNRDTRELFPDFGDAGTLCRDIFFGNNLIMRACGDHMVASPPLVVTRKEIDQMLGVAQRCVEEFEREIVRRGMV